European Patent Application EP 4 372 076 A1, published May 22, 2024. Title: Bis (2-hydroxyethyl) terephthalate (BHET) -degrading bacteria. Applicant: KEIO UNIVERSITY JEPLAN, INC. The sequence listing filed with the application follows.

SEQUENCE LISTING (3 sequences)

SEQ ID NO: 1 - DNA, 1458 bp, Delftia lacustris
attgaacgctggcggcatgccttacacatgcaagtcgaacggtaacaggtcttcggacgctgacgagtggcgaacgggtgagtaatacatcggaacgtgcccagtcgtgggggataactactcgaaagagtagctaataccgcatacgatctgaggatgaaagcgggggaccttcgggcctcgcgcgattggagcggccgatggcagattaggtagttggtgggataaaagcttaccaagccgacgatctgtagctggtctgagaggacgaccagccacactgggactgagacacggcccagactcctacgggaggcagcagtggggaattttggacaatgggcgaaagcctgatccagcaatgccgcgtgcaggatgaaggccttcgggttgtaaactgcttttgtacggaacgaaaaagctccttctaatacagggggcccatgacggtaccgtaagaataagcaccggctaactacgtgccagcagccgcggtaatacgtagggtgcgagcgttaatcggaattactgggcgtaaagcgtgcgcaggcggttatgtaagacagatgtgaaatccccgggctcaacctgggaactgcatttgtgactgcatggctagagtacggtagagggggatggaattccgcgtgtagcagtgaaatgcgtagatatgcggaggaacaccgatggcgaaggcaatcccctggacctgtactgacgctcatgcacgaaagcgtggggagcaaacaggattagataccctggtagtccacgccctaaacgatgtcaactggttgttgggaattagttttctcagtaacgaagctaacgcgtgaagttgaccgcctggggagtacggccgcaaggttgaaactcaaaggaattgacggggacccgcacaagcggtggatgatgtggtttaattcgatgcaacgcgaaaaaccttacccacctttgacatggcaggaagtttccagagatggattcgtgctcgaaagagaacctgcacacaggtgctgcatggctgtcgtcagctcgtgtcgtgagatgttgggttaagtcccgcaacgagcgcaacccttgtcattagttgctacattcagttgagcactctaatgagactgccggtgacaaaccggaggaaggtggggatgacgtcaagtcctcatggcccttataggtggggctacacacgtcatacaatggctggtacagagggttgccaacccgcgagggggagctaatcccataaaaccagtcgtagtccggatcgcagtctgcaactcgactgcgtgaagtcggaatcgctagtaatcgcggatcagcatgccgcggtgaatacgttcccgggtcttgtacacaccgcccgtcacaccatgggagcgggtctcgccagaagtaggtagcctaaccgcaaggagggcgcttaccacggcggggttcgtgactggggtgaag

SEQ ID NO: 2 - DNA, 1446 bp, Pseudarthrobacter sp.
gatgaacgctggcggcgtgcttaacacatgcaagtcgaacgatgatgcccacttgtgggtggattagtggcgaacgggtgagtaacacgtgagtaacctgcccttgactctgggataagcctgggaaactgggtctaataccggatatgactgactatcgcatggtggttggtggaaagcttttgcggttttggatggactcgcggcctatcagcttgttggtggggtaatggcctaccaaggcgacgacgggtagccggcctgagagggtgaccggccacactgggactgagacacggcccagactcctacgggaggcagcagtggggaatattgcacaatgggcggaagcctgatgcagcgacgccgcgtgagggatgacggccttcgggttgtaaacctctttcagtagggaagaagcgtaagtgacggtacctgcagaagaagcgccggctaactacgtgccagcagccgcggtaatacgtagggcgcaagcgttatccggaattattgggcgtaaagagctcgtaggcggtttgtcgcgtctgccgtgaaagtccggggctcaactccggatctgcggtgggtacgggcagactagagtgatgtaggggagactggaattcctggtgtagcggtgaaatgcgcagatatcaggaggaacaccgatggcgaaggcaggtctctgggcattaactgacgctgaggagcgaaagcatggggagcgaacaggattagataccctggtagtccatgccgtaaacgttgggcactaggtgtgggggacattccacgttttccgcgccgtagctaacgcattaagtgccccgcctggggagtacggccgcaaggctaaaactcaaaggaattgacgggggcccgcacaagcggcggagcatgcggattaattcgatgcaacgcgaagaaccttaccaaggcttgacatgaaccggaaacgcctggaaacaggtgccccacttgtggtcggtttacaggtggtgcatggttgtcgtcagctcgtgtcgtgagatgttgggttaagtcccgcaacgagcgcaaccctcgttctatgttgccagcacgtgatggtggggactcataggagactgccggggtcaactcggaggaaggtggggacgacgtcaaatcatcatgccccttatgtcttgggcttcacgcatgctacaatggccggtacaaagggttgcgatactgtgaggtggagctaatcccaaaaagccggtctcagttcggattggggtctgcaactcgaccccatgaagtcggagtcgctagtaatcgcagatcagcaacgctgcggtgaatacgttcccgggccttgtacacaccgcccgtcaagtcacgaaagttggtaacacccgaagccggtggcctaacccttttgggggggagccgtcgaaggtgggactggcgattgggactaag

SEQ ID NO: 3 - DNA, 1462 bp, Pseudomonas sp.
attgaacgctggcggcaggcctaacacatgcaagtcgagcggatgatgggagcttgctcccggattcagcggcggacgggtgagtaatgcctaggaatctgcctggtagtgggggacaacgtttcgaaaggaacgctaataccgcatacgtcctacgggagaaagcaggggaccttcgggccttgcgctatcagatgagcctaggtcggattagctagttggtggggtaaaggcctaccaaggcgacgatccgtaactggtctgagaggatgatcagtcacactggaactgagacacggtccagactcctacgggaggcagcagtggggaatattggacaatgggcgaaagcctgatccagccatgccgcgtgtgtgaagaaggtcttcggattgtaaagcactttaagttgggaggaagggcagtaagttaataccttgctgttttgacgttaccaacagaataagcaccggctaacttcgtgccagcagccgcggtaatacgaagggtgcaagcgttaatcggaattactgggcgtaaagcgcgcgtaggtggtttggtaagatggatgtgaaatccccgggctcaacctgggaactgcatccataactgcctgactagagtacggtagagggtggtggaatttcctgtgtagcggtgaaatgcgtagatataggaaggaacaccagtggcgaaggcgaccacctggactgatactgacactgaggtgcgaaagcgtggggagcaaacaggattagataccctggtagtccacgccgtaaacgatgtcgactagccgttgggatccttgagatcttagtggcgcagctaacgcgataagtcgaccgcctggggagtacggccgcaaggttaaaactcaaatgaattgacgggggcccgcacaagcggtggagcatgtggtttaattcgaagcaacgcgaagaaccttacctggccttgacatgtccggaatcttgcagagatgcgagagtgccttcgggaatcggaacacaggtgctgcatggctgtcgtcagctcgtgtcgtgagatgttgggttaagtcccgtaacgagcgcaacccttgtccttagttaccagcacgttatggtgggcactctaaggagactgccggtgacaaaccggaggaaggtggggatgacgtcaagtcatcatggcccttacggccagggctacacacgtgctacaatggtcggtacagagggttgccaagccgcgaggtggagctaatcccataaaaccgatcgtagtccggatcgcagtctgcaactcgactgcgtgaagtcggaatcgctagtaatcgtgaatcagaatgtcacggtgaatacgttcccgggccttgtacacaccgcccgtcacaccatgggagtgggttgctccagaagtagctagtctaaccgcaagggggacggttaccacggagtgattcatgactggggtgaag